European Patent Application EP 4 644 414 A1, published November 5, 2025. Title: MONOCLONAL ANTIBODY AGAINST CAPSID PROTEINS OF MULTIPLE AAV SEROTYPES, PREPARATION METHOD THEREFOR, AND USE THEREOF. Applicant: Nanjing GenScript Biotech Co., Ltd. The sequence listing filed with the application follows.

SEQUENCE LISTING (19 sequences)

SEQ ID NO: 1 - protein, 737 aa, synthetic construct
  source 1..737: note = rh.1 cap protein VP1
MAADGYLPDWLEDNLSEGIREWWALKPGAPKPKANQQKQDDGRGLVLPGYKYLGPFNGLDKGEPVNAADAAALEHGKAYDQQLQAGDNPYLRYNHADAEFQERLQEDTSFGGNLGRAVFQAKKRVLEPLGLVEEGAKTAPGKKRPVEPSPQRSPDSSTGIGKKGQQPARKRLNFGQTGDSESVPDPQPLGEPPAAPSGVGPNTMAAGGGAPMADNNEGADGVGNSSGNWHCDSTWLGDRVITTSTRTWALPTYNNHLYKQISNGTSGGSTNDNTYFGYSTPWGYFDFNRFHCHFSPRDWQRLINNNWGFRPKRLNFKLFNIQVKEVTTNEGTKTIANNLTSTVQVFTDSEYQLPYVLGSAHQGCLPPFPADVFMVPQYGYLTLNNGSQALGRSSFYCLEYFPSQMLRTGNNFQFSYTFEDVPFHSSYAHSQSLDRLMNPLIDQYLYYLVRTQTTGTGGTQTLAFSQAGPSSMANQARNWVPGPCYRQQRVSTTTNQNNNSNFAWTGAAKFKLNGRDSLMNPGVAMASHKDDEDRFFPSSGVLIFGKQGAGNDGVDYSQVLITDEEEIKATNPVATEEYGAVAINNQAANTQAQTGLVHNQGVIPGMVWQNRDVYLQGPIWAKIPHTDGNFHPSPLMGGFGLKHPPPQILIKNTPVPADPPLTFNQAKLNSFITQYSTGQVSVEIEWELQKENSKRWNPEIQYTSNYYKSTNVDFAVNTKGVYSEPRPIGTRYLTRNL

SEQ ID NO: 2 - protein, 600 aa, synthetic construct
  source 1..600: note = rh.1 cap protein VP2
MAPGKKRPVEPSPQRSPDSSTGIGKKGQQPARKRLNFGQTGDSESVPDPQPLGEPPAAPSGVGPNTMAAGGGAPMADNNEGADGVGNSSGNWHCDSTWLGDRVITTSTRTWALPTYNNHLYKQISNGTSGGSTNDNTYFGYSTPWGYFDFNRFHCHFSPRDWQRLINNNWGFRPKRLNFKLFNIQVKEVTTNEGTKTIANNLTSTVQVFTDSEYQLPYVLGSAHQGCLPPFPADVFMVPQYGYLTLNNGSQALGRSSFYCLEYFPSQMLRTGNNFQFSYTFEDVPFHSSYAHSQSLDRLMNPLIDQYLYYLVRTQTTGTGGTQTLAFSQAGPSSMANQARNWVPGPCYRQQRVSTTTNQNNNSNFAWTGAAKFKLNGRDSLMNPGVAMASHKDDEDRFFPSSGVLIFGKQGAGNDGVDYSQVLITDEEEIKATNPVATEEYGAVAINNQAANTQAQTGLVHNQGVIPGMVWQNRDVYLQGPIWAKIPHTDGNFHPSPLMGGFGLKHPPPQILIKNTPVPADPPLTFNQAKLNSFITQYSTGQVSVEIEWELQKENSKRWNPEIQYTSNYYKSTNVDFAVNTKGVYSEPRPIGTRYLTRNL

SEQ ID NO: 3 - protein, 534 aa, synthetic construct
  source 1..534: note = rh.1 cap protein VP3
MAAGGGAPMADNNEGADGVGNSSGNWHCDSTWLGDRVITTSTRTWALPTYNNHLYKQISNGTSGGSTNDNTYFGYSTPWGYFDFNRFHCHFSPRDWQRLINNNWGFRPKRLNFKLFNIQVKEVTTNEGTKTIANNLTSTVQVFTDSEYQLPYVLGSAHQGCLPPFPADVFMVPQYGYLTLNNGSQALGRSSFYCLEYFPSQMLRTGNNFQFSYTFEDVPFHSSYAHSQSLDRLMNPLIDQYLYYLVRTQTTGTGGTQTLAFSQAGPSSMANQARNWVPGPCYRQQRVSTTTNQNNNSNFAWTGAAKFKLNGRDSLMNPGVAMASHKDDEDRFFPSSGVLIFGKQGAGNDGVDYSQVLITDEEEIKATNPVATEEYGAVAINNQAANTQAQTGLVHNQGVIPGMVWQNRDVYLQGPIWAKIPHTDGNFHPSPLMGGFGLKHPPPQILIKNTPVPADPPLTFNQAKLNSFITQYSTGQVSVEIEWELQKENSKRWNPEIQYTSNYYKSTNVDFAVNTKGVYSEPRPIGTRYLTRNL

SEQ ID NO: 4 - protein, 118 aa, synthetic construct
  source 1..118: note = 5G4-1 VH
QSVKESEGGLFKPADTLSLTCTVSGFSLNNNDMSWVRQAPGNGLEYIGVMSSGGRLYAATWAKSRFTITRNTNLGTVTLKLTSLTAADTATYFCARGSPSSNRGIDIWGPGTLVTVSS

SEQ ID NO: 5 - protein, 108 aa, synthetic construct
  source 1..108: note = 5G4-1 VL
LTQTPSSVSAPVGGTVSINCQSDKSVYADNYLSWYQQTPGQPPKLLIYKASTLASGIPSRFKGSGSGTQFTLAISDVQCDDAATYYCAGGYSGNSDNGFGGGTEVVVR

SEQ ID NO: 6 - protein, 112 aa, synthetic construct
  source 1..112: note = 24F7-1 VH
QSLRESEGGLFKPADTLTLTCTVSGFSITAYNVGWVRQAPGKGLEWIGVIDISGATFYATWAKSRSTITRDTSLNTVTLKMTSLTAADTATYFCTRDPAFIWGPGTLVTVSS

SEQ ID NO: 7 - protein, 112 aa, synthetic construct
  source 1..112: note = 24F7-1 VL
DVVMTQTPASVEAAVGGTVTIKCQASQSVSSYLAWYQQKPGQPPKLLIYRASTLASGVPSRFKGSGSGTEFTLTISDLECADAATYYCQSYVYSNVLTYFNAFGGGTGVVVK

SEQ ID NO: 8 - protein, 5 aa, synthetic construct
  source 1..5: note = 5G4-1 VH CDR1
NNDMS

SEQ ID NO: 9 - protein, 16 aa, synthetic construct
  source 1..16: note = 5G4-1 VH CDR2
VMSSGGRLYAATWAKS

SEQ ID NO: 10 - protein, 11 aa, synthetic construct
  source 1..11: note = 5G4-1 VH CDR3
GSPSSNRGIDI

SEQ ID NO: 11 - protein, 13 aa, synthetic construct
  source 1..13: note = 5G4-1 VL CDR1
QSDKSVYADNYLS

SEQ ID NO: 12 - protein, 7 aa, synthetic construct
  source 1..7: note = 5G4-1 VL CDR2
KASTLAS

SEQ ID NO: 13 - protein, 11 aa, synthetic construct
  source 1..11: note = 5G4-1 VL CDR3
AGGYSGNSDNG

SEQ ID NO: 14 - protein, 5 aa, synthetic construct
  source 1..5: note = 24F7-1 VH CDR1
AYNVG

SEQ ID NO: 15 - protein, 16 aa, synthetic construct
  source 1..16: note = 24F7-1 VH CDR2
VIDISGATFYATWAKS

SEQ ID NO: 16 - protein, 5 aa, synthetic construct
  source 1..5: note = 24F7-1 VH CDR3
DPAFI

SEQ ID NO: 17 - protein, 11 aa, synthetic construct
  source 1..11: note = 24F7-1 VL CDR1
QASQSVSSYLA

SEQ ID NO: 18 - protein, 7 aa, synthetic construct
  source 1..7: note = 24F7-1 VL CDR2
RASTLAS

SEQ ID NO: 19 - protein, 14 aa, synthetic construct
  source 1..14: note = 24F7-1 VL CDR3
QSYVYSNVLTYFNA